European Patent Specification EP 3 628 060 B1, published May 7, 2025. Title: ASSAY FOR DETECTING HEPATITIS C VIRUS (HCV). Applicant: ABBOTT MOLECULAR INC. The sequence listing filed with the application follows.

SEQUENCE LISTING (26 sequences)

SEQ ID NO: 1 - DNA, 22 bp, Artificial Sequence
  Synthetic
atttgggcgtgcccccgcaaga

SEQ ID NO: 2 - DNA, 26 bp, Artificial Sequence
  Synthetic
cccggggcactcgcaagcaccctatc

SEQ ID NO: 3 - DNA, 17 bp, Artificial Sequence
  Synthetic
ccuugugguacugccug

SEQ ID NO: 4 - DNA, 18 bp, Artificial Sequence
  Synthetic
ctagccgagtagtgttgg

SEQ ID NO: 5 - DNA, 22 bp, Artificial Sequence
  Synthetic
atttgggcgtgcccccgcgaga

SEQ ID NO: 6 - DNA, 26 bp, Artificial Sequence
  Synthetic
cccggggcactcgtaagcaccctatc

SEQ ID NO: 7 - DNA, 26 bp, Artificial Sequence
  Synthetic
cccgaggcactcgcaagcaccctatc

SEQ ID NO: 8 - DNA, 26 bp, Artificial Sequence
  Synthetic
cccgaggcactcgtaagcaccctatc

SEQ ID NO: 9 - DNA, 26 bp, Artificial Sequence
  Synthetic
cccggggcactcgaaagcaccctatc

SEQ ID NO: 10 - DNA, 18 bp, Artificial Sequence
  Synthetic
ccttgtggtactgcctga

SEQ ID NO: 11 - DNA, 17 bp, Artificial Sequence
  Synthetic
ccuugtggtacugccug

SEQ ID NO: 12 - DNA, 17 bp, Artificial Sequence
  Synthetic
ccuugtgguacugccug

SEQ ID NO: 13 - DNA, 18 bp, Artificial Sequence
  Synthetic
ctagccgagtagtgttgg

SEQ ID NO: 14 - DNA, 18 bp, Artificial Sequence
  Synthetic
cuagccgaguagtguugg

SEQ ID NO: 15 - DNA, 28 bp, Artificial Sequence
  Synthetic
ctacagcagagttggcagcttcactttc

SEQ ID NO: 16 - DNA, 22 bp, Artificial Sequence
  Synthetic
gtctggcctttcagcaagtttc

SEQ ID NO: 17 - DNA, 24 bp, Artificial Sequence
  Synthetic
acgagttcatgagggcaggccgct

SEQ ID NO: 18 - DNA, 20 bp, Artificial Sequence
  Synthetic
gctccatcttagccctagtc

SEQ ID NO: 19 - DNA, 26 bp, Artificial Sequence
  Synthetic
agcactctctgcagtcatgcggctca

SEQ ID NO: 20 - DNA, 19 bp, Artificial Sequence
  Synthetic
cggctagctgtgaaaggtc

SEQ ID NO: 21 - DNA, 21 bp, Artificial Sequence
  Synthetic
cggctagctgtgaaaggtccg

SEQ ID NO: 22 - DNA, 17 bp, Artificial Sequence
  Synthetic
ccuugugguacugccug

SEQ ID NO: 23 - DNA, 17 bp, Artificial Sequence
  Synthetic
ccuugtggtacugccug

SEQ ID NO: 24 - DNA, 17 bp, Artificial Sequence
  Synthetic
ccuugtgguacugccug

SEQ ID NO: 25 - DNA, 18 bp, Artificial Sequence
  Synthetic
ctagccgagtagtgttgg

SEQ ID NO: 26 - DNA, 18 bp, Artificial Sequence
  Synthetic
cuagccgaguagtguugg